European Patent Specification EP 3 862 436 B1, published August 28, 2024. Title: Method for predicting or prognosticating the response to the treatment of multiple sclerosis with interferon beta. Applicant: Servicio Andaluz de Salud Universidad de Málaga. The sequence listing filed with the application follows.

SEQUENCE LISTING (4 sequences)

SEQ ID NO: 1 - DNA, 2479 bp, Artificial Sequence
  sIFNAR2 nucleotide sequence
  misc_feature (1)..(2479)
agatgtaaaagtcaagagaagactctaaaaatagcaaagatgcttttgagccagaatgccttcatcttcagatcacttaatttggttctcatggtgtatatcagcctcgtgtttggtatttcatatgattcgcctgattacacagatgaatcttgcactttcaagatatcattgcgaaatttccggtccatcttatcatgggaattaaaaaaccactccattgtaccaactcactatacattgctgtatacaatcatgagtaaaccagaagatttgaaggtggttaagaactgtgcaaataccacaagatcattttgtgacctcacagatgagtggagaagcacacacgaggcctatgtcaccgtcctagaaggattcagcgggaacacaacgttgttcagttgctcacacaatttctggctggccatagacatgtcttttgaaccaccagagtttgagattgttggttttaccaaccacattaatgtgatggtgaaatttccatctattgttgaggaagaattacagtttgatttatctctcgtcattgaagaacagtcagagggaattgttaagaagcataaacccgaaataaaaggaaacatgagtggaaatttcacctatatcattgacaagttaattccaaacacgaactactgtgtatctgtttatttagagcacagtgatgagcaagcagtaataaagtctcccttaaaatgcaccctccttccacctggccaggaatcagaattttcataactttttagcctggccatttcctaacctgccaccgttggaagccatggatatggtggaggtcatttacatcaacagaaagaagaaagtgtgggattataattatgatgatgaaagtgatagcgatactgaggcagcgcccaggacaagtggcggtggctataccatgcatggactgactgtcaggcctctgggtcaggcctctgccacctctacagaatcccagttgatagacccggagtccgaggaggagcctgacctgcctgaggttgatgtggagctccccacgatgccaaaggacagccctcagcagttggaactcttgagtgggccctgtgagaggagaaagagtccactccaggacccttttcccgaagaggactacagctccacggaggggtctgggggcagaattaccttcaatgtggacttaaactctgtgtttttgagagttcttgatgacgaggacagtgacgacttagaagcccctctgatgctatcgtctcatctggaagagatggttgacccagaggatcctgataatgtgcaatcaaaccatttgctggccagcggggaagggacacagccaacctttcccagcccctcttcagagggcctgtggtccgaagatgctccatctgatcaaagtgacacttctgagtcagatgttgaccttggggatggttatataatgagatgactccaaaactattgaatgaacttggacagacaagcacctacagggttctttgtctctgcatcctaacttgctgccttatcgtctgcaagtgttctccaagggaaggaggaggaaactgtggtgttcctttcttccaggtgacatcacctatgcacattcccagtatggggaccatagtatcattcagtgcattgtttacatattcaaagtggtgcactttgaaggaagcacatgtgcacctttcctttacactaatgcacttaggatgtttctgcatcatgtctaccagggagcagggttccccacagtttcagaggtggtccaggaccctatgatatttctcttctttcgttcttttttttttttttttgagacagagtctcgttctgtcgcccaagctggagcgcaatggtgtgatcttggctcactgcaacatccgcctcccgggttcaggtgattctcctgcctcagcctccctcgcaagtagctgggattacaggcgcctgccaccatgcctagcaaatttttgtatttttagtggagacaggattttaccatgttggccaggctggtctcgaactcctgacctcaagtgatctgccctcctcagcctcgtaaagtgctgggattacaggggtgagccgctgtgcctggctggccctgtgatatttctgtgaaataaattgggccagggtgggagcagggaaagaaaaggaaaatagtagcaagagctgcaaagcaggcaggaagggaggaggagagccaggtgagcagtggagagaaggggggccctgcacaaggaaacagggaagagccatcgaagtttcagtcggtgagccttgggcacctcacccatgtcacatcctgtctcctgcaattggaattccaccttgtccagccctccccagttaaagtggggaagacagactttaggatcacgtgtgtgactaatacagaaaggaaacatggcgtcggggagagggataaaacctgaatgccatattttaagttaaaaaaaaaaaa

SEQ ID NO: 2 - protein, 239 aa, Artificial Sequence
  sIFNAR2 amino acid sequence
  PEPTIDE (1)..(239)
MLLSQNAFIFRSLNLVLMVYISLVFGISYDSPDYTDESCTFKISLRNFRSILSWELKNHSIVPTHYTLLYTIMSKPEDLKVVKNCANTTRSFCDLTDEWRSTHEAYVTVLEGFSGNTTLFSCSHNFWLAIDMSFEPPEFEIVGFTNHINVMVKFPSIVEEELQFDLSLVIEEQSEGIVKKHKPEIKGNMSGNFTYIIDKLIPNTNYCVSVYLEHSDEQAVIKSPLKCTLLPPGQESEFS

SEQ ID NO: 3 - protein, 331 aa, Artificial Sequence
  Primary antibody
  PEPTIDE (1)..(331)
MLLSQNAFIVRSLNLVLMVYISLVFGISYDSPDYTDESCTFKISLRNFRSILSWELKNHSIVPTHYTLLYTIMSKPEDLKVVKNCANTTRSFCDLTDEWRSTHEAYVTVLEGFSGNTTLFSCSHNFWLAIDMSFEPPEFEIVGFTNHINVMVKFPSIVEEELQFDLSLVIEEQSEGIVKKHKPEIKGNMSGNFTYIIDKLIPNTNYCVSVYLEHSDEQAVIKSPLKCTLLPPGQESESAESAKIGGIITVFLIALVLTSTIVTLKWIGYICLRNSLPKVLRQGLTKGWNAVAIHRCSHNALQSETPELKQSSCLSFPSSWDYKRASLCPSD

SEQ ID NO: 4 - protein, 331 aa, Artificial Sequence; identical to SEQ ID NO: 3
  Secondary antibody
  PEPTIDE (1)..(331)